European Patent Application EP 4 269 425 A1, published November 1, 2023. Title: Novel trigonal glucagon/GLP-1/GIP receptor agonist and use thereof. Applicant: HANMI PHARM. CO., LTD. The sequence listing filed with the application follows.

SEQUENCE LISTING (36 sequences)

SEQ ID NO: 1 - protein, 40 aa, Artificial Sequence
  Trigonal agonist
  MISC_FEATURE (2): Xaa is aminoisobutyric acid (Aib)
  MISC_FEATURE (16)..(20): amino acids at positions 16 and 20 form a ring
YXQGTFTSDYSKYLDEQRAKEFVQWLLDHHPSSGQPPPSC

SEQ ID NO: 2 - protein, 40 aa, Artificial Sequence
  Trigonal agonist
  MISC_FEATURE (2): Xaa is aminoisobutyric acid (Aib)
  MISC_FEATURE (16)..(20): amino acids at positions 16 and 20 form a ring
YXQGTFTSDYSKYLDEQAAKEFVQWLLDHHPSSGQPPPSC

SEQ ID NO: 3 - protein, 40 aa, Artificial Sequence
  Trigonal agonist
  MISC_FEATURE (2): Xaa is aminoisobutyric acid (Aib)
  MISC_FEATURE (16)..(20): amino acids at positions 16 and 20 form a ring
YXQGTFTSDYSKYLDEQRAKEFIAWLLDHHPSSGQPPPSC

SEQ ID NO: 4 - protein, 40 aa, Artificial Sequence
  Trigonal agonist
  MISC_FEATURE (2): Xaa is aminoisobutyric acid (Aib)
  MISC_FEATURE (16)..(20): amino acids at positions 16 and 20 form a ring
YXQGTFTSDYSIYLDEQRAKEFIAWLLAHHPSSGQPPPSC

SEQ ID NO: 5 - protein, 40 aa, Artificial Sequence
  Trigonal agonist
  MISC_FEATURE (2): Xaa is aminoisobutyric acid (Aib)
  MISC_FEATURE (16)..(20): amino acids at positions 16 and 20 form a ring
YXQGTFTSDYSKYLDEKRAKEFVQWLLDQHPSSGQPPPSC

SEQ ID NO: 6 - protein, 40 aa, Artificial Sequence
  Trigonal agonist
  MISC_FEATURE (2): Xaa is aminoisobutyric acid (Aib)
  MISC_FEATURE (16)..(20): amino acids at positions 16 and 20 form a ring
YXQGTFTSDYSKALDEKAAKDFVQWLLDQHPSSGQPPPSC

SEQ ID NO: 7 - protein, 40 aa, Artificial Sequence
  Trigonal agonist
  MISC_FEATURE (2): Xaa is aminoisobutyric acid (Aib)
  MISC_FEATURE (16)..(20): amino acids at positions 16 and 20 form a ring
YXQGTFTSDYSKALDEKAAKDFVQWLKDQHPSSGQPPPSC

SEQ ID NO: 8 - protein, 39 aa, Artificial Sequence
  Trigonal agonist
  MISC_FEATURE (2): Xaa is aminoisobutyric acid (Aib)
  MISC_FEATURE (16)..(20): amino acids at positions 16 and 20 form a ring
YXQGTFTSDCSKYLDEKAAKEFVQWLLDHHPSSGQPPPS

SEQ ID NO: 9 - protein, 39 aa, Artificial Sequence
  Trigonal agonist
  MISC_FEATURE (2): Xaa is aminoisobutyric acid (Aib)
  MISC_FEATURE (12)..(16): amino acids at positions 16 and 20 form a ring
YXEGTFTSDYSEYMEKEAVREFICWLVKGGPSSGAPPPS

SEQ ID NO: 10 - protein, 40 aa, Artificial Sequence
  Trigonal agonist
  MISC_FEATURE (2): Xaa is aminoisobutyric acid (Aib)
  MISC_FEATURE (16)..(20): amino acids at positions 16 and 20 form a ring
YXQGTFTSDYSKYLDERASKDFVQWLLDHHPSSGQPPPSC

SEQ ID NO: 11 - protein, 40 aa, Artificial Sequence
  Trigonal agonist
  MISC_FEATURE (2): Xaa is aminoisobutyric acid (Aib)
  MISC_FEATURE (16)..(20): amino acids at positions 16 and 20 form a ring
YXQGTFTSDYSIYLDEKAAKEFVQWLLDQHPSSGQPPPSC

SEQ ID NO: 12 - protein, 40 aa, Artificial Sequence
  Trigonal agonist
  MISC_FEATURE (2): Xaa is aminoisobutyric acid (Aib)
  MISC_FEATURE (20): Xaa is aminoisobutyric acid (Aib)
YXEGTFTSDYSIQLDKQAAXAFVQWLIAGGPSSGAPPPSK

SEQ ID NO: 13 - protein, 12 aa, HOMO SAPIENS
ESKYGPPCPSCP

SEQ ID NO: 14 - protein, 11 aa, Artificial Sequence
  Variant of hinge region
ESKYGPPPSCP

SEQ ID NO: 15 - protein, 11 aa, Artificial Sequence
  Variant of hinge region
ESKYGPPCPSP

SEQ ID NO: 16 - protein, 10 aa, Artificial Sequence
  Variant of hinge region
ESKYGPPCPS

SEQ ID NO: 17 - protein, 10 aa, Artificial Sequence
  Variant of hinge region
ESKYGPPCPP

SEQ ID NO: 18 - protein, 8 aa, Artificial Sequence
  Variant of hinge region
KYGPPCPS

SEQ ID NO: 19 - protein, 8 aa, Artificial Sequence
  Variant of hinge region
ESKYGPPC

SEQ ID NO: 20 - protein, 7 aa, Artificial Sequence
  Variant of hinge region
EKYGPPC

SEQ ID NO: 21 - protein, 6 aa, Artificial Sequence
  Variant of hinge region
ESPSCP

SEQ ID NO: 22 - protein, 5 aa, Artificial Sequence
  Variant of hinge region
EPSCP

SEQ ID NO: 23 - protein, 4 aa, Artificial Sequence
  Variant of hinge region
PSCP

SEQ ID NO: 24 - protein, 10 aa, Artificial Sequence
  Variant of hinge region
ESKYGPPSCP

SEQ ID NO: 25 - protein, 9 aa, Artificial Sequence
  Variant of hinge region
KYGPPPSCP

SEQ ID NO: 26 - protein, 9 aa, Artificial Sequence
  Variant of hinge region
ESKYGPSCP

SEQ ID NO: 27 - protein, 8 aa, Artificial Sequence
  Variant of hinge region
ESKYGPPC

SEQ ID NO: 28 - protein, 7 aa, Artificial Sequence
  Variant of hinge region
KYGPPCP

SEQ ID NO: 29 - protein, 7 aa, Artificial Sequence
  Variant of hinge region
ESKPSCP

SEQ ID NO: 30 - protein, 6 aa, Artificial Sequence
  Variant of hinge region
ESPSCP

SEQ ID NO: 31 - protein, 4 aa, Artificial Sequence
  Variant of hinge region
EPSC

SEQ ID NO: 32 - protein, 3 aa, Artificial Sequence
  Variant of hinge region
SCP

SEQ ID NO: 33 - protein, 221 aa, homo sapiens
PSCPAPEFLGGPSVFLFPPKPKDTLMISRTPEVTCVVVDVSQEDPEVQFNWYVDGVEVHNAKTKPREEQFNSTYRVVSVLTVLHQDWLNGKEYKCKVSNKGLPSSIEKTISKAKGQPREPQVYTLPPSQEEMTKNQVSLTCLVKGFYPSDIAVEWESNGQPENNYKTTPPVLDSDGSFFLYSRLTVDKSRWQEGNVFSCSVMHEALHNHYTQKSLSLSLGK

SEQ ID NO: 34 - protein, 442 aa, Homo sapiens
  MISC_FEATURE (1)..(442): Amino acids at position 1 to 442 form Human Immunoglobulin G4 Fc Fragment (homodimer)
  MISC_FEATURE (1)..(221): Amino acids at position 1 to 221 form one monomer
  MISC_FEATURE (222)..(442): Amino acids at position 222 to 442 form one monomer
  DISULFID (3)..(224): Amino acids at position 3 and position 224 form an inter-disulfide bond
  DISULFID (35)..(95): Amino acids at position 35 and position 95 form an intra-chain disulfide bond
  DISULFID (141)..(199): Amino acids at position 141 and position 199 form an intra-chain disulfide bond
  DISULFID (256)..(316): Amino acids at position 256 and position 316 form an intra-chain disulfide bond
  DISULFID (362)..(420): Amino acids at position 362 and position 420 form an intra-chain disulfide bond
PSCPAPEFLGGPSVFLFPPKPKDTLMISRTPEVTCVVVDVSQEDPEVQFNWYVDGVEVHNAKTKPREEQFNSTYRVVSVLTVLHQDWLNGKEYKCKVSNKGLPSSIEKTISKAKGQPREPQVYTLPPSQEEMTKNQVSLTCLVKGFYPSDIAVEWESNGQPENNYKTTPPVLDSDGSFFLYSRLTVDKSRWQEGNVFSCSVMHEALHNHYTQKSLSLSLGKPSCPAPEFLGGPSVFLFPPKPKDTLMISRTPEVTCVVVDVSQEDPEVQFNWYVDGVEVHNAKTKPREEQFNSTYRVVSVLTVLHQDWLNGKEYKCKVSNKGLPSSIEKTISKAKGQPREPQVYTLPPSQEEMTKNQVSLTCLVKGFYPSDIAVEWESNGQPENNYKTTPPVLDSDGSFFLYSRLTVDKSRWQEGNVFSCSVMHEALHNHYTQKSLSLSLGK

SEQ ID NO: 35 - protein, 4 aa, Artificial Sequence
  partial sequecne of the trigonal agonist (X27-X30)
LDHH

SEQ ID NO: 36 - protein, 4 aa, Artificial Sequence
  partial sequecne of the trigonal agonist (X27-X30)
LDQH